European Patent Application EP 4 414 375 A1, published August 14, 2024. Title: Peptide having anti-inflammatory activity and use thereof. Applicant: CAREGENE CO., LTD. The sequence listing filed with the application follows.

SEQUENCE LISTING (9 sequences)

SEQ ID NO: 1 - protein, 4 aa, synthetic construct
TWNS

SEQ ID NO: 2 - DNA, 21 bp, synthetic construct
  source 1..21: mol_type = other DNA
aacatccaaccttcccaaacg

SEQ ID NO: 3 - DNA, 21 bp, synthetic construct
  source 1..21: mol_type = other DNA
gaccctaagcccccaattctc

SEQ ID NO: 4 - DNA, 20 bp, synthetic construct
  source 1..20: mol_type = other DNA
ggaacggtatccacggatgt

SEQ ID NO: 5 - DNA, 20 bp, synthetic construct
  source 1..20: mol_type = other DNA
gaggtacatcacgtgggaag

SEQ ID NO: 6 - DNA, 20 bp, synthetic construct
  source 1..20: mol_type = other DNA
tgagtggtagccagcaaagc

SEQ ID NO: 7 - DNA, 20 bp, synthetic construct
  source 1..20: mol_type = other DNA
ctgcagtccaggttcaatgg

SEQ ID NO: 8 - DNA, 20 bp, synthetic construct
  source 1..20: mol_type = other DNA
ttcgacacatgggataacga

SEQ ID NO: 9 - DNA, 20 bp, synthetic construct
  source 1..20: mol_type = other DNA
tctttcaacacgcaggacag